European Patent Specification EP 3 240 898 B1, published August 14, 2024. Title: Prenylcysteine oxidase 1 inhibitors for the prevention and/or treatment of oxidative stress-related degenerative diseases and prenylcysteine oxidase 1 as diagnostic marker. Applicant: Centro Cardiologico Monzino S.p.A. - IRCCS. The sequence listing filed with the application follows.

SEQUENCE LISTING (16 sequences)

SEQ ID NO: 1 - DNA, 23087 bp, Homo sapiens
gcgcagccgcgcagcggtgggaggactgcggggctcttgaggccagctgcagagcttgtggaggccatggggcgcgtcgtcgcggagctcgtctcctcgctgctggggttgtggctgttgctgtgcagctgcggatgccccgagggcgccgagctgcgtgctccgccagataaaatcggtaggcgagaagggggcggcgcgggaaggtgctggagcgcgccccgcgccgggcggccgctgcgcagtgcgcccagatcccacagccgcgacgcagtccagcggtgcaggccgagccagctgcgcaggtcgcgctttcccccattcacacttcagggcggctttcagctctggtcggaataggactgtgcattcccaggcgtggagaggtgcccacttgaggaatgggcgtggacggggacaggggcgggcgggcaggcaggcgcctagcgtacctgtagcccctgtctcttaggtgtggggctccggggaggcctaggtttctctatcttcccgttgaacactgaccgtgaagactccagtgttctggcttgacctggggcgcccggccagattaacaggctcacgcaggcacagcacagggaggagtgcaaacaagttgaccctgcctgcttcccttgggaggctgaaccgccttcccccagctccgctttgctgaggtcggcctgctctcagaggcccttggcttgcacagtttctccgcctaggactaacacagctgcagaaagaatctgttctctttccactgtcaagagctccagtgtcaggagccttggctctttgcttcctgtctccctcccgcccccctttaaagttgtgttcttcggtatcattaacctatctacattgaatctagacacaacaaagctaggcataaatggccgtcactttattaaaaatgcgtgctggaaaggtccacctctaatgtgcccgtgagttgggcatctggaagggtgtgcaggccccttggttcctccataaagacctgtgagaatctttgggcatctggaaaaaaaatcgagttaatgtcaatatgttaattaatctactgcttttgtctgggaacagtgtctgtccagattcagggagttagaccttcgctgcaggtgtcactcttcccccaccaaattgttggtaatagctttgagtaacaacctctgctattgatggtctttcaaaaacaaaacaactcacagagctggtaaaaggggaaaatataatcttctgtttttttccctcatagcgattattggagccggaattggtggcacttcagcagcctattacctgcggcagaaatttgggaaagatgtgaagatagacctgtttgaaagagaagaggtcgggggccgcctggctaccatgatggtgcaggggcaagaatacgaggcaggaggttctgtcatccatcctttaaatctgcacatgaaacgttttgtcaaagacctgggtatgtaattttggtcttggagctcaccagattactgtgtgacatccccggatatttttatcagatggagaactgaaatttctgccttgttaattgccttacagagacgttggtaaaactgttttcctcactttcttgttagttggtactgcctgagttaggagcagttctgctgtaatgggacactagttgtctgtatcttcagttatctggaattacagccatggggtgggggtgggaatggctgccattgtctttttttttcttttgaggagtttcgctcttgtcgctcaggctggagtgcaatggtgcgatcttggctcactgcaacctctgcctcccgggttcaagcgattctcctgccttagcctcctgagtagctgggattacaggtgcctgccaccacgcccagctaatttttgtattttcagtagtgacggggtttcaccatgttggccagctggtcttgaactcctgacctcaggtgatccgcctgccttggccttccaaagtgctgggattacaggggtgagccaccgtgcccggcctctgttgtctgttcttaaaattctgggtttgtgttaaagaatcagagaaggtttggagatagtcatctcattgtgatcattttgcagctgagtaaatgagacccagagacttgaattgtctggctcaaagtcactcacatatggccatggccagggtcagtggctcatgcctgtaatcccagcactttgggaggccgaggcagaggatcacttgagcccaggagttagaaaccagtctgggcaacatagtgagatcctgtctttactaaaaataaaaaagttagcctggtgtgatggcacaaacctgtagtcccagcttcttgggaggcagaggcaggaggatcccttgagcctgggagatagaagctgcagtgagccttgcatgccactgcactccagcctgggcaacaaagtgagaccctatcaaaacaaaccaccaccaacaaaacaaactccgtcacacagctgtggatgcagacacgtgcctagaacttgggatgtgcaactgctgccctgacagcagaggagctggataggtcatggggaaagtctgacaggcctctggaggccctttcggcagggagtattttgtaactttggcctccttccagttatctgaaatatccagttttgcaaaataggattctcacaggaatggaagtgcctcagctgccttccacatcctctgtagatgctgcctctgcttccgtttcctccacgagggcgaaggtatacccagaacaaattatgccacgaagatgcatgtctgacatctttgtttttaaattgaattcagttggtactctggcttttttcctttgactatccagtttttttagacttttagtctaaaaatagccaggtaaaaatatatctacttttgatatattaatatttacatgatcatctgacccatcgcctagcaaatctgcttttggacagtgtagtgaaagtatagtgtttcacactgttccaaagatagagctcctttatgtgtctcctgagaactgagggaagccccaaattcactcagattacgttctttcatttgatcagcatagacaccactgacttagctgtgctttatgtttttgcaggtctctctgctgttcaggcctctggtggcctactggggatatataatggagagactctggtatttgaggagagcaactggttcataattaacgtgattaaattagtttggcgctatggatttcaatccctccgtatgcacatgtgggtagaggacgtgttagacaagttcatgaggtaattttttttccttccatttaacctaagatcttttaatttaggttaaattaaacttgatgaactttaggaattatgatttcttgtaagcattttctacctcacagcaaggcctgtttataacattgttaggcaaaatgttttgtagaaactatgcagactatttgcttggatattgaaaggttggtttatttttgcttctgaagtgtattttgcaaatgcttctttagtgttgccagatactgttagatgccttgaattcttatgacaacttactctggtaggtactgtttttagcttctttaaacagatgcagaaggtggcggtgtagagaggttttaaaaggcaagttcacccacatagtaagtggtatagctggagttgccacccaggcagtctggcctttgagtcttcactcttaatctctatgctgtgctggtgttgtgtatatgaattgagataatgtgtacaagagcttgtagaaaggatcagaaaacttaaatggcctttaatagtgacatgttttcagtgaaccagcagcctgaagtagagtaaaagttccatattccaagaatttacattctagcactgttttgggtagtgagaattcaggtgcctctttttcgtccttatgcttttctatatttaaacagtttttttaatgcgtgtgaatatgtatcactttggtaatcaggaagactaacataaaatagccagtctaattttgaaaggtacaatctgtatttttaaagctgttggcatgttctagttttttagtttttttgtttttttgtttttgagatggagtttcgcttgttgcctaggctggagtgcaatggttcgatattggctcactgcaacctctgcctcttgggttcaagcgatactcctgcctcaggctcccgagtagctgggattacagatgcctgccaccacgcccagctaatttttgtatttttagtagagatggggtttcaccctcttggccaggctggtctcgaactcctgacctcaggtgatccacctgcctcggcctcccaaagtgctgggattacaggtgtgagctaccgagcttggccggcatgtgctaattttttttttttttttttttgagatggagttttgctctgtcgcccgggctggagtgcagtggcaccatctcggctcactgcaacctctgcctccctggttcaagcgattctcctgcctcagactcccgaatagctgggattacaggtgcctgccactgtgcctggctaattttttgtatttttagtagagacggggtttcactgtgttagccaggatggtcttgatctcctgacctcgtgatccgcctgcctcagcctcccaaagtgttgggattgcaggcatgagccactgtgcccggctagcacatgctaatttttatgctgctttacagttttaggtactggaggccaggatcgcatcattacactccagcctgggtgacagaacaagattccatcttgaggggaaaaacaaaacaaaacaaaacatgtcatatgaccaggtattgaacaggacaaatatgagttaagcagggctgggcacagtggcttatgcctctaatcccagaattttgggaggctgaggctggtggatcacctgaggtcaggagtttgagaccagcctgaccaacatggtaaaaccctgtctctacaaaaaatataaaaatttagccggcgtggtggtgcatgcctgtaatcccagctacttgtgagcctgaggcaggagaatcacttgaacctgggaggcagaggttgcagtgagccacgatcgtgccattacactctagcctgggggacagagccagactgtctaaaaaaaaaaaaaagaaagctaagcaggatatgctctggtttctataactcatggtagtttggggtttctttctttctcaacatcattcttaggtcagttccttaaatgcctttcccgtgggtaccttaagtccatctacagtgcataatgtttttaagtagccattcattcattcacccaatattgaatacctgttaggtgctaggcattgttctatgttgagagtataggacctacaacatgtccttgtcctcaaagaatatatattctagtggagagacaggcaatacacaaccaaggaaatatatagaatttgcgtagagacggccagtcactttatagaaggtgggtggcatggtgctgcatactcagcaggcagatcaagttctgatggcatcagccctgcttgtgtgtattgtttttcttttcttttcttttttttttttgagatagagtctcgttttgtcgcccaggctggagtgcagtggcgggatctcggcttactgcaacatctgcctcccaggttcaagtgattctcctgcctcagcctcctgagtagctgggactacaggcacatgccaccatgcctggttaattttttgtatttttagtagagatgtggtttcaccgtgttagccaggctggtctcaaactcctgaccttgtgatctgcctgtctcggcttcccaaagtgttgggattataggcgtgagccactgtgcccggccctcttttttttttttttttttttgatacaggtctcactctgtcacccaggctggagtgcagtggtgtgatcatggctcactgcagcctggacctcctgggctcaggggatctgcctaccttagcctctgtgtagctgggactacaggcacgtgccatcagatctggctaattttttgtattttttttgtagagatgaggtttggccatgttgcccaggctggtcttgaattcctgggctcgagtgttccactcacctgggcctcccaaagtgttgggattacggttgtgagctcctgttcccagccttgtttttttttttatctgtggcttgcttgagatgtagagaattgccctttgagaaattaagaaattacttttttttttttgagatgagtttcactctgtcacccaggctggagtgcagtggtgcaatctcggctcactgcaacctctgcctcctgagtccaagcgattctcctgcctcagcctcctgagtagctgggattacaggcatgtgccaccatacccagataatttttttatttttagtagagatggggttttaccatgttggctaggctggtctcaaactcctggccttaattgatctgcccgccttggcctcctaaagtgctgcgattacaggcatgagccaccgcacctggcctaagaaatcacttttgaagtgaattcaaggtattacagaactgggaaaaagaaccagtgaggggatacataggttatactgtttttgactttaaaaaataatttacgggccgggcgcggtggcacacgcctgtaatcccagcactttgggaggccaaggcagatagatcttgaggtcaggagttcgagaccagcctggccaacatggtgaaactccgccttgctaaaaatacaaaaattagctgggtgtggaggcgcagctaatgccagctacttgggaggctgaggcagtagaatcgcttgaacccaggaagcggaggttgtggtgagccaagatcaaagtatacacaaggtggagaaagacctatgtaacagtagtaaaccatgacactcgaaagagggctcaagcttgtggtaggcaatactcgaaaacagtgcattcattcattctctgctgttggaggtacttgagtggaaatcctgcagcccctgacatcagcactagctagcttaatttccacttctgcacatacatttatgtagttgttctggttggatgccattcttaactaattttttttttttttttttttttgagaccaagtcttgctccgtcacccaggctggagtacggtggtgcaatcacagctcactgcagctttgacctcctggtctcaagtcatcttccagcctcagctgggactataggcatgtgccatcatgcttggctaattttttaaatttttgtagagacagggtgttgccatgttgcccaagctgatcttgaactcctgggctcaagtgatcctcccaccttggcctcccaaagtgttgggattacaggcgtgagccaccgcgctcagccggatgccattctttactcccaagtccaacctcttatctcactttttcagcaaagcatttccttaatgcttcaatcaacattcatctttcttttcaaacatcccttattatacggtgcacactgtgtgcttgtgttctatgctacgcacagtaactagaatgtagtagatgtttactcagatgtttgtggaatttaaatctctggtctgctgatggcttcctgttgagatatcttggcttgtagactaggttaaagcttattcttctctctcaagttagtgcatttctggggacttgtaagatccttaacacttcttgatctgagactgatagactcacagggaaaggctttataaacaccctttcttccttccagttactcctaccaaatattttgagtcaatttttgttctttcatttcccaaacccactctatcttgaatcccatcagcctttaaaatacatccagtattccactacttctctccaggattactgctaccactttgttccaagtcaccaccactgtctcttgtctggattgctagagtagcctcctattataggctgaataatcctctcccctgctgtctgccacaagatgtccatgtcttaattcctggaacctgtgaatgtgttaccttttgaggtaaaagagacgttgcagatatggttaaggatgggtagattattctggattatctaggtgggcccaatataatcacaagggtccttagagaggcaggaggatcagggtaggtagtaggagatgtgatgatggaaggaagagattggagtgatgctaggaaggggtgtgcgtccacgagccaaggaatgcaggtggcctgtagaggctggaaaagacagtcttccctcagagcttctagaaggaaccagccttgtgcacaccttgattttagcccggagagactgactttggtcttctaatttacagaaccgtaagattataactttttttttttttgttagtatttattaatcattcttgggtgttcttcggagagggggatttggcagggtcataggacaatagtggagggaaggtcagcggataaacatgtgaacaaaggtctctggttttcctaggcagagggccctgccgccttccgcagtgtttgtgtccctgggtacttgagattagggagtggtgatgactcttaacgagtatgctgccttcaagcatctgtttaacaaagcacatcttgcaccgcccttaatccatttaacccttagtggacacagcacatgtttcagagagcatggggttgggggtaaggtcatagataaacagcattccaaggcagaagaatttctcttactacagaacaaaatggagtctcctatgtccacctctttctacacagacacagtaacaatccgatctctccttcctttccccacatttcccccacttctattcgacaaaactgccatcgtcatcatggcccgttctcaatgagctattgggtacacctcccagacggggtggcggctgggcagaggggctcctcacttcccagacagggcggctgctgggcggaggggctcctcacttctcagagagggcggctggtcagagaggctcctcacctcccagacgggatggcggcggggcagagacactcctcagttcccagacggcgtcgcggccgggcagaggcgctcttcacatctcagacggggcggcggggcagaggcgctccccacatcccagacgatgggcagccgggcagagacgctcctcacttcctagacgggatgacggccgggaagaggcgctcctcacttcccagactgggcggccgggcagaggagttcctcacatcccagacgatgggcggccaggcaaagacactcctcacttcctagacggggtggcggctgggcagaggctgcaatctcagcacttttgggaggtcaaggcaggcggctgggaggtggaggttgtagcgagccgagatcacgccactgcactccagcctgggcaacattgagcactgagtgagcgacactccgtctgcaatcctggcacctcgggaggccgaggctggcagatcactcatggtcaggaactggagaccagcccggccaacacggtgaaaccccgtctccaccaaaaaatacgaaaaccagtcaggcgtggcggcgcgcgcctgcaatcccaggcacttggcaggctgaagcaggagaatcaggcagggaggttgcagtgagtcgagatggcagcagtacagtccagccttggctcggcatcagagggagaccgtggagagggagagggggagggggagggggagagggagagctgttttttgttttgagacagagtcttgctctgtcacccaggctggagtgcagtggcacaatcttggctcactgcagcctccgcctcctgggttcaagcagttctctgcctcagcctcccgagtagttgggatcacaggcgcccaccaccatgcccggctaatttttgtatttttagtagagatggggtttcaccatcttggccaggcaggtcttgcactcctgacctcgtgatccacccgcctcagcctcccaaagtgctgggattacaggtgtgagccactgcacccggccgtaaatttgtgttgttttaagccactaagtttgtggtaatttgttatagcagcagtggaaaaccaagacacctcctaaatcatctgccattactgttatattgctaccatttgttctcaggttagcagccaaagtagttctttaaaatctaaggctcatcacatcactccactaactcagaaaccttcagtggctatttcattaatagagatttatagccaaaatctgttttgtgactgagaagacatgacaggattctgtgctctcatcccttacttttaaatttgttttccccaaaattcataggttgaaacactagccacccagtactcagaatgtgactgcatatgtatgtagggcctttaaatatgtgattaagttaaaatgaggtctttagcgtagaccctaaaacaatttgatgggtgtccttaagattaggacacagaaaggaggccaaggcgggcagatcacctgaggttgggagttcgagaccagcctgaccaacatggtgaaaccccttctctactaaaaatacaaaaaattagctgggcgtggtggtgcatgcttgtaatcccagctactcaggaaggctgaggcaagagaatcacttgaacctgggcggcagaggttgcagtgagccattgcactccagcctgggcaacaagcgtgaaactctgtctcagaaaaaaaaaaaaaaaaattgggacacagaagaaacacacaaagaccatgtgaggacacagcaagaaggtggccatctgcaagccaaggaaataggcctcagaagaaaccgaatgcatccacaccttgatcttggacttttggcctacagaactataagaaataaaactttttttgtttaagccatccagtctttggtactgtgttatggcagtcttggtgaactaatacactgttgtcattttcagtaactgtccattattgaaaatgggatattgaagtctccattattgttgaactatgtatttcagttctgtcaagatcatttgatcatattcatgaaggtttatttctgggttttcttatttgtttcaaggatctgtgtgtctgtttttttttttttttcagatgatgttttactctgttgcccaggctagagtgtagtatgttcacagcaacctctgcctcccaggctcaagcaattctccaacctcaggccccttgagtggctgggactacagatgtgcactaccatgcccagctaatttttttttttttttttttgagacagagtctcgctctgttgcccaggctggagttcagtggcgctatctcggctcactgcaacctctgcctcccgggttcaagcaattcttgtgcctcagcctcctgagtaggtgggactacaggcatgcaccaccaaccctggctaattttttgtgtttttagtagagatgggttttcgccatgatggccaggctggtctcgaactcctaacctcaagtgatcctccagcctgtgcctcccaatgtgctgggattacaggcgtgagccactgcacccggccttttttaaaaagtttttttggtcagcctcttgtagtctctattgatgtcatagcctccggcatctgtgatgttaaacaattgccacagattttttttttgacacgtggacacgtgccctcaggatggggctgttgcatagagtgaactttgaatcaggtcgaataaagacaagccttcaggatagagctttttcggagctgccagataggtcaaatattgacagttctctgaggatagtgctttttgggagctacaaactcgttgtgttctctccagtggcttctagcttgctagtttcacattgcagttggaagggtgctggttttattttttatttttttttctctctctctttttctctttctttctttctttcgacggagtctccctcttgtcgcccaggctggagtgcaatggtgcgatcttggctcactgcaacctccatctcctgggttcaagcgattctcctgcctcagcctcctgaatagctgggattacaggcgtgtgccaccacacctggctaattttttatatttttggtacagatggtgtttcaccatgttgggcaggctggtcttgaactcctgacctcaagtgatccgcctggctcagcttcccagagtgctgggattacaggtgtgagccaccatgcctgccagacatttttcttgaataaatactccttggacttggaaaggctttggtttatctgcagagctctgaaagagtcaatgttgatcatttttggcagtattctcatagcttttatggaggagcagatttccagaggtccttcctctgccattctggaagtttcctctccccagtaacatttctggctgtaccactcccggttctcccatatcactctgcttcagctgctctggcttcattgtttcttgaatgtgccaggcaagcttctgtcatgtgacctttgcattgcttttacctctaccggaaatattttcccccaggtgtttgcctggtttgcatcctcatctccttcgggtctttggtctatatcatcttctcagtgaggcttttcctgaccactcttgtttttggacagtcttatttagaattcaaccctcctaaccccatgtatttctagtcttcttttcagaccattttctccttttttttttcttttgagatggagtctgtctctgttgcccaggctggagtgcagtggcacgatcttggctctcctcggctcaccttggctcactgtgccactgcaccactacgcccggctaattttgtatttttagtagagacagggtttctccatgttggtcaggctggtctcgaactcctgacctcaggtgatccacctgtcttggcctcccaaagtgctgggattacaggcgtgagccactgtgcctggccccagttatatttttttaaaaattattatttttttgtttttgtttttgttttttttaagacaaggtctcactctgttgcccaagctggatggagtgcagtggtgtgatcacagctcactgcagcctcaaccagcggggctgaagtgatcctcatgcctcagcttcctgaatagctgggactacaggcatgcctcaccatgcctggctaatttttttttttttttttttctgtaagtattttatttatcactgaagaaaaaacacagcagcaagttctgtgttggcttcaatgagaccaaatagttcatctttaacatagctactgcgctccaaaattgaagtcaacacagtcattactacaaattacttgttgaaagaatctatcttcaaaagaaagaaaattaggaaagagaatttaaacgattcctccaaaccatacatttataaatattgtcatatttaaaatgcttgaaaggcgtgaattctccattaatggaaaagcagtttgctattggcaacagaaaaaaactcagcgataatttaccaaatgctttaaaatttaaaagctatactgtttggattcacacttgcgcagtaatcttgtcattacaacaactgcaaattgctttgtactcaccttctctcaagtaaaatctaaagaaaaccccaccgtatccaatgtttgtaatgtttacttcaagtgaatctaaaaaatttctaaatttagtttatggtaaatacctcaaaatacctaaaaataggtacgtatcaaccacttaagggtgtgaaaattgtttcagattcactgctttaaagggtcttcaaatatattttctttaacagaaccttacttcattccaaattattatcagatatttcaaaataaaaaaaaagtatcagttctataccaagataaaggtgttactcaatacctgaaggttcacattttaaatttattttttagtttttcttttttgtcaacaaatgattgatgaaataatgcaacacccttaaattccagaaaatggcatggtttttccaacctcctgtggatatggtgcatgatcaatctattatataggagcctggctaatttttaatttttttttttttttttttgagagggagtttcactctgtcaccaaggctagagtgcagtggcacgatctcggctcactgcaacctctacctcccaggttcaagcgattctcctgcctccacctcccaagtagctggtattacaggcatgcgccaccatgcccagttaatttttgtatttttagtagaggtggggtttcgctatgttggccaggctggtctcaaactcctgacctcaagcgatctgcccgcctcagcctcccaaagtgctgggattacaggcatgaaccactgcgcctggctaatttttacattttgtgtacagacagagtcttgctatgttgcccaggctagtcttgaactcctggcctcaaggtatcctcctgtcttactctgtcacccaggctggagtatattggctggctgttcacaggtgcaaccataatgtactacagccttgtgcccctgggcttaagtgatcctcccacctcagcctcttgagtagctgtgactacaggtgcatgctgcctcacctgggtgctgttttttagtagtatttattctgttttttcatttattattattatttttttgagatggagtcttgctctgtcatccagggtgtagtgcagtggtgtgatcttgacttactgcaacctctgtctcctgggtcaagcaattctcatgcctcagccacctgagtagctgggattacaggcatgcaccaccacacctggataatttttgtatttttagtagagatggggtttcaccatgttggccaggcggtctcaaactactgacctcaagtgatgctgccccactttgcctcccaaagtgctaggattacaggcatgagccaccatacccagcagtgtatttattctaatacgattagttgtatcatgaaacaattagagtgctctctgtttatattgtgtatatagtttcatctcaccgctgccaccccgccccctcccagggagacttgcttgagtgaggttgcagctctggcaggagcagttggggaatatgttttttatagcatcattagtagcttatttaattgactgttattttctcatgttgaccattagccaaagatcactcttctttggatatgagatatccaggctattatttttctgaagaattcagtgtttccatcctactttttccagtctcctaaagactgggacccaaatgctatggttagaaggtatttagtttctcagttttggcatagatatcgaatcagtttttccaataaaaatgtgtttaacattttgtacacttatactactactatgcttttagtaggtaatactgaaatggttataatactgtcccttgttctgtaaaaaaatatagtacattttgagagaaaaacttgatgtgaaagtttcccttccatgatcagtgatagggatctttccttggctcttaatttcttattttcatatacttatctctgcatgtgccttattacttatccctaactataagccccttaagggaataagagataaaccccgtattacttatcccaaacttaagcctgttttccatctttgtactatttgcaacatgaaaaattgtgtttgaattactgaatgcactaatttatgtgaatgttgttttaaatccataaaatgcagagaagtgttgggtgatatttttctttttggtcaagtgatgttttctaaaaaataatagaaagcatctaattgttgaatgagtggcattggtgctaagttttatgaggcttctggagatgatataactgtggactgggaagttgagcaagacttttcagagaaggtgggattcaagttctgttaaggaagaatagatgttccatggttaggaatgggaagtgtattcaggttggagggaagagcttgtgcactggtggggatacagcatgtagggcaaatttagagaccagtgaatgggtcaggtgtgctccagtggagactgtgcatgtgtgggtgattgacagcagagtgggcaagttgtgattgagccttatacttgccatgtggcctttagacaaagtattttacttctacttttttttttttttttttttgagatggagtctcgctctgttgcccaggctggagtgcagcggtgtgatctcggctcactgcaacctccgctttctgggttgaagcgattctcctgcctcagcctcctgaatagctgggattacaggcgtgcgccaccaggcccagctaatttttgtatttttagtagagacggggtttcaccatgttggtcaggctggtctcaaactcctgacctagtgatctgcctgccttggccttccaaagagctaggattacaggcatgaaaccaccgcgcctggccttacttctactttttatttttcctttttcttcttctttctttcttccttagtttcttttctttttttttttctttttttttttttaagagacactgtcactgtctggcccaggctggagtgcagcggcattatcacagttcactgcggccttgaattccggggctcaagcagtcctcctgcctcagcctcccaagtagctgggaccacaggcatacaccactatgcctggttaatttttgtatttttagtaaagctggggttttgccatgttggccaggctggtcttgaactcctgacctcaggtgacctgcccacctctgcctcccaaagtgtggggattataggcgtgagccactgcacctagatgtcagtttgattcttatgacgccacttcccttctttatacatccccttccccacatcttgtttggtatttaatggatttctcttcttttccaaaggatctaccgctaccagtctcatgactatgccttcagtagtgtcgaaaaattacttcatgctctaggaggagatgacttccttggaatgcttaatcgaacacttcttgaaaccttgcaaaaggccggcttttctgagaagttcctcaatgaaatgattgctcctgttatgagggtcaattatggccaaagcacggacatcaatgcctttgtgggtaagccagggcttgaaacagtggtggacattagttcacagaggggcttacctgatgctatggtggttcctgactttaggctgtggattggaggctacttttctctgtgaacctcagacattgttagcaaaattgtgcgtatgtagatgtgcatttttagggggagagggtctttagctttcattagttcagtaattcttaactgggggagattttgctcccaggggccatttagcaatgtctagagacatttggagtagaacatgtaattgggaagggagagtgggtagagagcctcttacaaaaagtcagaattaaaacacatttttcctcctattgacaggggcggtgtcactgtcctgttctgattctggcctttgggcagtagaaggtggcaataaacttgtttgctcagggcttctgcaggcatccaaaagcaatcttatatctggctcagtaatgtacatcgaggagaaaacaaagaccaagtacacaggtaagcttgaatttcttattgttcctgatatcccctgcagaaaatgattgctcagggagaaacacttctcttctgtcatctcttactcagttctaaaatgatgaaacttgaaattgtatatattgtaccatatagaaatattccccaatgggccaggcacggtggctcatgcctgtaatccctgtactttgggaggccaaggagggtggatcacctgaggtcaggagatcaagactagcctggccaacatagttaaaccctgtctctactaaaaatacaaaaaattagccgggcgtggtggcaggtgcctgtaatcccagctactcgggaggctgaggcaggagaatcacatgaacccagggggcagaggttgcagtgagccaagatcacaccactgcactctagcctgggtgacggagtgagactccatctaaaaaaaaaaaaaaaaaaaaaaaattccccagtgtagttaagtgctgtggcatcactccttggatttgaaaaataatcttttttttttttgagatggagtctcgctcttttgcccaggccggactgtagtggcctatctcggctcactgcaagctccgcctcccgggttcacgccattctcctgcctcagcgtcccgagtagctgggactataggcgcctgcctcagcgtcccgagtagctgggactataggcgcctgccaccgcgctcggctaattttttgtatttttagtagagacggggtttcaccatgttagccaggatggtctcgatctcctgacctcgtgatccacccacctcggcctcccaaagtgctgagattacaggtgtgagccaccatgcccggccgaaagataatcttaccttcaaaagtaaaaattctgtattttgtacttactgacattctgaataagaaattggcctcaatgtaataaaaatgcaagggacaactatcttaagggatataacttcttcaattctttagaattatagagaaattatgaagaaggtatacaattatttttagaaggtatgttagaaacactaaacaaatatatgcctccttatttcctctaggaaatccaacaaagatgtatgaagtggtctaccaaattggaactgagactcgttcagacttctatgacatcgtcttggtggccactccgttgaatcgaaaaatgtcgaatattacttttctcaactttgatcctccaattgaggaattccatcaatattatcaacatatagtgacaactttagttaagggggaattgaatacatctatctttagctctagacccatagataaatttggccttaatacagttttaaccactgataattcagatttgttcattaacagtattgggattgtgccctctgtgagagaaaaggaagatcctgagccatcaacagatggaacatatgtttggaagatcttttcccaagaaactcttactaaagcacaaattttaaagctctttctgtcctatgattatgctgtgaagaagccatggcttgcatatcctcactataagcccccggagaaatgcccctctatcattctccatgatcgactttattacctcaatggcatagagtgtgcagcaagtgccatggagatgagtgccattgcagcccacaacgctgcactccttgcctatcaccgctggaacgggcacacagacatgattgatcaggatggcttatatgagaaacttaaaactgaactatgaagtgacacactcctttttcccctcctagttccaaatgactatcagtggcaaaaaagaacaaaatctgagcagagatgattttgaaccagatattttgccattatcattgtttaataaaagtaatccctgctggtcataggaaaacacacggttctaattaagtgtgaaggtatagctattgcacttatgccatctccaaaatttcttaagtattctttcactatccattaggagtttttcttaaacttgtctgataataagaatcacctggagttaggaggtggtggttgcagtgagccaatctcaccattgcacttcagcctgagcaacacgagcaaaactccgtctcaaaagtaaataaaaataatcacctggagtttgttaaaccatatggattctcaagctcctctcttgaagattctgattcagtaggtctgggagtggcgcgctggattttgatcaaaattgtagagcattttaaggtgagtacctgagggagaacttaaagacatcttagttggggagtagtccttttgaattttacagctagatataatcttcagtcagataaaatttatgggagctggtgtcttatgcctgactcttagtaatttcataccggtttgaagtacgtgtgcccatgcctaaagccttgactttcagaatgttgtcttttgattcttctgtcttgatttgattaggggtgaaatttagaagtcttagtaatgtaacttgaagatgttaaacaaaaatctcaagtaaaatgaaaagcaaatatgggctactgaattaagaaactggcattctagtattaaatcctcacttcaggagcttttaaaaatactgagacccccccataaccagagattcagattcaaagactgaggataggaccttagcattgtagctatttaaagtttctaatgtgcacccagggttgggaatcaccaatgtgggtgtgaaaatgcctacaaagggttttagtgccttagaagtcctaagaagcccaatctgtatcaaagcagatccattttgcaaggatctttcttttagaactttctcagttctcttagtaagaactttagaagtaatcttgataataagcacagacagcctaacagcagaggcaacttaaataactcctgagcagttggcactagaacagaatacttggaatgacaccaaagttaaccaagtccagcatatgtccaaagagttaagtgtttcatttactgtagcattctgggtgagaaattggttgctgaaatcttaagacagtggtctcaaccttggctgcacattggaatcacctgtagggttttaaagcatccaaatggtaattaacaggcagcaaaacttcagaactagttctgcatctactgtgcaaagatcatgattaactgtcaagacactggtagaacagaacaagcaaaagattaagagttcaaaagtaaatgcaaccaatttaacatgtagtgttattaaaaaattacaaaggcctagaccagcctgggcaacatggtgaaaccccatctctacaaaaaatttttaaaaagttggccaggcatggtaatgcgcgcctgtggtcccagctgctcgggaggctgaggtgggaggatcacttgagccttggaggtcaaggctgcagtgaatcatgatcatgccactgtactccagcctgggcaacagagaccatcttaaaaaaaaaaaatccttccattgaatagaaacttcaaagtccttcatcagatcatggcattagctactttagcaaaatagtgtaaactttggttctgagtaaaaatgacttcttccctaccacagttgtgaatgttaatatgctgataaaactgccaagatatatttgataggtaggggattaaactcatggtttgtcaaaagagtgtttttttctagttttattcttaacagatatgttgaggtattcatatttgtttccttttgtggttttaatgaagacaatttgtaaagtaatactgttatgtatatgctaaatgttggtaaatactaattaatttccatcatttgtagacttgttttgcaatgggatatatttttacttataataccaatttaggctgggcgcagtggctcacgcctgtaatcccagcactttgggaggccaaggcaaacggatcacgaggtcaggagatcaagaccatcctggccaacatggtgaaaccccatctctactgaatacacaaaaattggctggacatggtggcgcatgtctgtaatcccagctactgtaatctcagctacttgggaggctgaggcaggagaattgcctcaaccgggaggcggaggttgcagtgagccaagatcgcaccactgcactccagcctggcaacagagcgagactctgtctcagaaaaaaaaaacaaaaaccagtttaggctgggtatggtggctcaccagcactttgggaggctgaggcaggtggatctcttgaggtcgggagtttgagaccagcctggccaacatggtgaaaccctgtctttactaaaaatacaaaaattagccaggcatggtggcgtgtgccagtaatcccagctacttgggaggctgaggcgcgagaatcgcttgaaccctggagatggaggttgcagtgagcagagatcgcaccactgcactccagcctgggcaagagtgagactgtgtctcaaaaggaaaaaaaaaaaattaaaaatgttgctggtattacatcaaacctactctggataaattttccagtagggcatctgaaattgctttggcaaaagcaaaacaggttatcaatacaccaaggacatcaagtagttttaatgcaactacagtgttgagtgcttttttactgggagaaaaatcctagcagaacctgctactctgggcgcattaggtagttttatgcaactatagtattaagagttttattggaagaaaaaacactgtcagagcttactgctccagacctttttttttaatagaagagactggtaaaaatgatgcaggggctgaatgaaagccagctctgctccagtggctctctgagttgagcatgcatcagttaccttaagggcttgttaaaacatcgctaggctccaccctgtttattcaataagtttgttatgggatataagaagatgcattttattaagttccccagtgatgctgctgttctactataggaaccacacttgaagaactagttctacaattcagctgtatgttgtaaaggagtcaagtcaatgaaggagttataaagagttgctgaaaaatggagtaacagtgtatgggacttcacatcagttctccttattgattgttagtttgatccctcttgttcttttgttgtaaacattttctataattaggaaatgccatttaagagtgagagaggtatatatctatgagccattgtgtttggtgttttacaagaactttaccatactggtgtgtagtccattctgtacagtttaaaagtgattcacgatttgcaggctttttatcagatcacaaaaaaatcagtctttaagcatttgcttggtaaggtttcttaagattaggtttataatacaaccatctgtaatgtatctctcgtttgagcttgtgggccatacaattcattaactagatgaatacattgtggacagcatcctcactacccctctctactcactcacaaagaaccatgatacactggaatgtttttctctggaatcctctttctactcttgtattaaaatttttccccacttcatgattatattcaaaataaacaactacatcatta

SEQ ID NO: 2 - DNA, 5377 bp, Homo sapiens
gcgcagccgcgcagcggtgggaggactgcggggctcttgaggccagctgcagagcttgtggaggccatggggcgcgtcgtcgcggagctcgtctcctcgctgctggggttgtggctgttgctgtgcagctgcggatgccccgagggcgccgagctgcgtgctccgccagataaaatcgcgattattggagccggaattggtggcacttcagcagcctattacctgcggcagaaatttgggaaagatgtgaagatagacctgtttgaaagagaagaggtcgggggccgcctggctaccatgatggtgcaggggcaagaatacgaggcaggaggttctgtcatccatcctttaaatctgcacatgaaacgttttgtcaaagacctgggtctctctgctgttcaggcctctggtggcctactggggatatataatggagagactctggtatttgaggagagcaactggttcataattaacgtgattaaattagtttggcgctatggatttcaatccctccgtatgcacatgtgggtagaggacgtgttagacaagttcatgaggatctaccgctaccagtctcatgactatgccttcagtagtgtcgaaaaattacttcatgctctaggaggagatgacttccttggaatgcttaatcgaacacttcttgaaaccttgcaaaaggccggcttttctgagaagttcctcaatgaaatgattgctcctgttatgagggtcaattatggccaaagcacggacatcaatgcctttgtgggggcggtgtcactgtcctgttctgattctggcctttgggcagtagaaggtggcaataaacttgtttgctcagggcttctgcaggcatccaaaagcaatcttatatctggctcagtaatgtacatcgaggagaaaacaaagaccaagtacacaggaaatccaacaaagatgtatgaagtggtctaccaaattggaactgagactcgttcagacttctatgacatcgtcttggtggccactccgttgaatcgaaaaatgtcgaatattacttttctcaactttgatcctccaattgaggaattccatcaatattatcaacatatagtgacaactttagttaagggggaattgaatacatctatctttagctctagacccatagataaatttggccttaatacagttttaaccactgataattcagatttgttcattaacagtattgggattgtgccctctgtgagagaaaaggaagatcctgagccatcaacagatggaacatatgtttggaagatcttttcccaagaaactcttactaaagcacaaattttaaagctctttctgtcctatgattatgctgtgaagaagccatggcttgcatatcctcactataagcccccggagaaatgcccctctatcattctccatgatcgactttattacctcaatggcatagagtgtgcagcaagtgccatggagatgagtgccattgcagcccacaacgctgcactccttgcctatcaccgctggaacgggcacacagacatgattgatcaggatggcttatatgagaaacttaaaactgaactatgaagtgacacactcctttttcccctcctagttccaaatgactatcagtggcaaaaaagaacaaaatctgagcagagatgattttgaaccagatattttgccattatcattgtttaataaaagtaatccctgctggtcataggaaaacacacggttctaattaagtgtgaaggtatagctattgcacttatgccatctccaaaatttcttaagtattctttcactatccattaggagtttttcttaaacttgtctgataataagaatcacctggagttaggaggtggtggttgcagtgagccaatctcaccattgcacttcagcctgagcaacacgagcaaaactccgtctcaaaagtaaataaaaataatcacctggagtttgttaaaccatatggattctcaagctcctctcttgaagattctgattcagtaggtctgggagtggcgcgctggattttgatcaaaattgtagagcattttaaggtgagtacctgagggagaacttaaagacatcttagttggggagtagtccttttgaattttacagctagatataatcttcagtcagataaaatttatgggagctggtgtcttatgcctgactcttagtaatttcataccggtttgaagtacgtgtgcccatgcctaaagccttgactttcagaatgttgtcttttgattcttctgtcttgatttgattaggggtgaaatttagaagtcttagtaatgtaacttgaagatgttaaacaaaaatctcaagtaaaatgaaaagcaaatatgggctactgaattaagaaactggcattctagtattaaatcctcacttcaggagcttttaaaaatactgagacccccccataaccagagattcagattcaaagactgaggataggaccttagcattgtagctatttaaagtttctaatgtgcacccagggttgggaatcaccaatgtgggtgtgaaaatgcctacaaagggttttagtgccttagaagtcctaagaagcccaatctgtatcaaagcagatccattttgcaaggatctttcttttagaactttctcagttctcttagtaagaactttagaagtaatcttgataataagcacagacagcctaacagcagaggcaacttaaataactcctgagcagttggcactagaacagaatacttggaatgacaccaaagttaaccaagtccagcatatgtccaaagagttaagtgtttcatttactgtagcattctgggtgagaaattggttgctgaaatcttaagacagtggtctcaaccttggctgcacattggaatcacctgtagggttttaaagcatccaaatggtaattaacaggcagcaaaacttcagaactagttctgcatctactgtgcaaagatcatgattaactgtcaagacactggtagaacagaacaagcaaaagattaagagttcaaaagtaaatgcaaccaatttaacatgtagtgttattaaaaaattacaaaggcctagaccagcctgggcaacatggtgaaaccccatctctacaaaaaatttttaaaaagttggccaggcatggtaatgcgcgcctgtggtcccagctgctcgggaggctgaggtgggaggatcacttgagccttggaggtcaaggctgcagtgaatcatgatcatgccactgtactccagcctgggcaacagagaccatcttaaaaaaaaaaaatccttccattgaatagaaacttcaaagtccttcatcagatcatggcattagctactttagcaaaatagtgtaaactttggttctgagtaaaaatgacttcttccctaccacagttgtgaatgttaatatgctgataaaactgccaagatatatttgataggtaggggattaaactcatggtttgtcaaaagagtgtttttttctagttttattcttaacagatatgttgaggtattcatatttgtttccttttgtggttttaatgaagacaatttgtaaagtaatactgttatgtatatgctaaatgttggtaaatactaattaatttccatcatttgtagacttgttttgcaatgggatatatttttacttataataccaatttaggctgggcgcagtggctcacgcctgtaatcccagcactttgggaggccaaggcaaacggatcacgaggtcaggagatcaagaccatcctggccaacatggtgaaaccccatctctactgaatacacaaaaattggctggacatggtggcgcatgtctgtaatcccagctactgtaatctcagctacttgggaggctgaggcaggagaattgcctcaaccgggaggcggaggttgcagtgagccaagatcgcaccactgcactccagcctggcaacagagcgagactctgtctcagaaaaaaaaaacaaaaaccagtttaggctgggtatggtggctcaccagcactttgggaggctgaggcaggtggatctcttgaggtcgggagtttgagaccagcctggccaacatggtgaaaccctgtctttactaaaaatacaaaaattagccaggcatggtggcgtgtgccagtaatcccagctacttgggaggctgaggcgcgagaatcgcttgaaccctggagatggaggttgcagtgagcagagatcgcaccactgcactccagcctgggcaagagtgagactgtgtctcaaaaggaaaaaaaaaaaattaaaaatgttgctggtattacatcaaacctactctggataaattttccagtagggcatctgaaattgctttggcaaaagcaaaacaggttatcaatacaccaaggacatcaagtagttttaatgcaactacagtgttgagtgcttttttactgggagaaaaatcctagcagaacctgctactctgggcgcattaggtagttttatgcaactatagtattaagagttttattggaagaaaaaacactgtcagagcttactgctccagacctttttttttaatagaagagactggtaaaaatgatgcaggggctgaatgaaagccagctctgctccagtggctctctgagttgagcatgcatcagttaccttaagggcttgttaaaacatcgctaggctccaccctgtttattcaataagtttgttatgggatataagaagatgcattttattaagttccccagtgatgctgctgttctactataggaaccacacttgaagaactagttctacaattcagctgtatgttgtaaaggagtcaagtcaatgaaggagttataaagagttgctgaaaaatggagtaacagtgtatgggacttcacatcagttctccttattgattgttagtttgatccctcttgttcttttgttgtaaacattttctataattaggaaatgccatttaagagtgagagaggtatatatctatgagccattgtgtttggtgttttacaagaactttaccatactggtgtgtagtccattctgtacagtttaaaagtgattcacgatttgcaggctttttatcagatcacaaaaaaatcagtctttaagcatttgcttggtaaggtttcttaagattaggtttataatacaaccatctgtaatgtatctctcgtttgagcttgtgggccatacaattcattaactagatgaatacattgtggacagcatcctcactacccctctctactcactcacaaagaaccatgatacactggaatgtttttctctggaatcctctttctactcttgtattaaaatttttccccacttcatgattatattcaaaataaacaactacatcatta

SEQ ID NO: 3 - protein, 505 aa, Homo sapiens
MGRVVAELVSSLLGLWLLLCSCGCPEGAELRAPPDKIAIIGAGIGGTSAAYYLRQKFGKDVKIDLFEREEVGGRLATMMVQGQEYEAGGSVIHPLNLHMKRFVKDLGLSAVQASGGLLGIYNGETLVFEESNWFIINVIKLVWRYGFQSLRMHMWVEDVLDKFMRIYRYQSHDYAFSSVEKLLHALGGDDFLGMLNRTLLETLQKAGFSEKFLNEMIAPVMRVNYGQSTDINAFVGAVSLSCSDSGLWAVEGGNKLVCSGLLQASKSNLISGSVMYIEEKTKTKYTGNPTKMYEVVYQIGTETRSDFYDIVLVATPLNRKMSNITFLNFDPPIEEFHQYYQHIVTTLVKGELNTSIFSSRPIDKFGLNTVLTTDNSDLFINSIGIVPSVREKEDPEPSTDGTYVWKIFSQETLTKAQILKLFLSYDYAVKKPWLAYPHYKPPEKCPSIILHDRLYYLNGIECAASAMEMSAIAAHNAALLAYHRWNGHTDMIDQDGLYEKLKTEL

SEQ ID NO: 4 - protein, 13 aa, Homo sapiens
YQSHDYAFSSVEK

SEQ ID NO: 5 - protein, 11 aa, Homo sapiens
  MISC_FEATURE (3)..(3): Cysteine is carbamidomethylated
LVCSGLLQASK

SEQ ID NO: 6 - DNA, 57 bp, Artificial Sequence
  Hairpin sequence:
gatccggaaagatgtgaagatagattcaagagatctatcttcacatctttccttttt

SEQ ID NO: 7 - DNA, 21 bp, Artificial Sequence
  siRNA
ggaaagaugugaagauagatt

SEQ ID NO: 8 - DNA, 21 bp, Artificial Sequence
  siRNA
ucuaucuucacaucuuucctt

SEQ ID NO: 9 - DNA, 57 bp, Artificial Sequence
  Hairpin sequence
gatccccactccgttgaatcgaaattcaagagatttcgattcaacggagtggttttt

SEQ ID NO: 10 - DNA, 21 bp, Artificial Sequence
  siRNA
ccacuccguugaaucgaaatt

SEQ ID NO: 11 - DNA, 21 bp, Artificial Sequence
  siRNA
uuucgauucaacggaguggtt

SEQ ID NO: 12 - DNA, 57 bp, Artificial Sequence
  Hairpin sequence
gatccgaagcccaatctgtatcaattcaagagattgatacagattgggcttcttttt

SEQ ID NO: 13 - DNA, 21 bp, Artificial Sequence
  siRNA
gaagcccaaucuguaucaatt

SEQ ID NO: 14 - DNA, 21 bp, Artificial Sequence
  siRNA
uugauacagauugggcuuctt

SEQ ID NO: 15 - protein, 13 aa, Artificial Sequence
  Y-13-K heavy peptide
  MISC_FEATURE (13)..(13): (13C6; 15N2)
YQSHDYAFSSVEK

SEQ ID NO: 16 - protein, 11 aa, Artificial Sequence
  L-11-R heavy peptide
  MISC_FEATURE (3)..(3): Cysteine is carbamidomethylated
  MISC_FEATURE (11)..(11): (13C6; 15N2)
LVCSGLLQASK